European Patent Application EP 4 631 976 A1, published October 15, 2025. Title: ANTI-CD155 ANTIBODY AND USE THEREOF. Applicant: HEFEI TG IMMUNOPHARMA CO., LTD. Application CN. The sequence listing filed with the application follows.

SEQUENCE LISTING (81 sequences)

SEQ ID NO: 1 - protein, 8 aa, synthetic construct
GYTFTSSY

SEQ ID NO: 2 - protein, 8 aa, synthetic construct
IYAGTGDT

SEQ ID NO: 3 - protein, 14 aa, synthetic construct
ARHGYTGRGWYFAV

SEQ ID NO: 4 - protein, 8 aa, synthetic construct
TGAVTTSN

SEQ ID NO: 5 - skipped

SEQ ID NO: 6 - protein, 9 aa, synthetic construct
ALWYSNKFV

SEQ ID NO: 7 - protein, 8 aa, synthetic construct
GYTFTSSY

SEQ ID NO: 8 - protein, 8 aa, synthetic construct
IYAGTGDT

SEQ ID NO: 9 - protein, 14 aa, synthetic construct
ARHGYTGRGWYFAV

SEQ ID NO: 10 - protein, 8 aa, synthetic construct
TGAVTTSN

SEQ ID NO: 11 - skipped

SEQ ID NO: 12 - protein, 9 aa, synthetic construct
ILWYSNHFV

SEQ ID NO: 13 - protein, 8 aa, synthetic construct
GYTFTSSY

SEQ ID NO: 14 - protein, 8 aa, synthetic construct
IYAGTGDT

SEQ ID NO: 15 - protein, 14 aa, synthetic construct
ARHGLTGRHWYFAV

SEQ ID NO: 16 - protein, 8 aa, synthetic construct
TGAVTTSN

SEQ ID NO: 17 - skipped

SEQ ID NO: 18 - protein, 9 aa, synthetic construct
ILWYSNKFV

SEQ ID NO: 19 - protein, 8 aa, synthetic construct
GYTFTSSY

SEQ ID NO: 20 - protein, 8 aa, synthetic construct
IYAGTGDT

SEQ ID NO: 21 - protein, 14 aa, synthetic construct
ARHGMTGRGWYFAV

SEQ ID NO: 22 - protein, 8 aa, synthetic construct
TGAVTTSN

SEQ ID NO: 23 - skipped

SEQ ID NO: 24 - protein, 9 aa, synthetic construct
ILWYSNKFV

SEQ ID NO: 25 - protein, 121 aa, synthetic construct
QVQLVQSGAEVKKPGASVKVSCKASGYTFTSSYISWVRQAPGQGLEWIAWIYAGTGDTNYNQKFTGRVTMTTDTSTSTAYMELRSLRSDDTAVYYCARHGYTGRGWYFAVWGQGTTVTVSS

SEQ ID NO: 26 - protein, 109 aa, synthetic construct
QAVVTQEPSLTVSPGGTVTLTCRSSTGAVTTSNLANWVQQKPGQAFRGLIGHTNNRAPGVPARFSGSLLGDKAALTLSGAQPEDEAEYYCALWYSNKFVFGGGTKLTVL

SEQ ID NO: 27 - protein, 121 aa, synthetic construct; identical to SEQ ID NO: 25

SEQ ID NO: 28 - protein, 109 aa, synthetic construct
QAVVTQEPSLTVSPGGTVTLTCRSSTGAVTTSNYANWVQQKPGQAFRGLIGGTNNRAPGVPARFSGSLLGDKAALTLSGAQPEDEAEYYCILWYSNHFVFGGGTKLTVL

SEQ ID NO: 29 - protein, 121 aa, synthetic construct
QVQLVQSGAEVKKPGASVKVSCKASGYTFTSSYISWVRQAPGQGLEWIAWIYAGTGDTNYNQKFTGRVTMTTDTSTSTAYMELRSLRSDDTAVYYCARHGLTGRHWYFAVWGQGTTVTVSS

SEQ ID NO: 30 - protein, 109 aa, synthetic construct
QAVVTQEPSLTVSPGGTVTLTCRSSTGAVTTSNIANWVQQKPGQAFRGLIGGTNNRGPGVPARFSGSLLGDKAALTLSGAQPEDEAEYYCILWYSNKFVFGGGTKLTVL

SEQ ID NO: 31 - protein, 121 aa, synthetic construct
QVQLVQSGAEVKKPGASVKVSCKASGYTFTSSYISWVRQAPGQGLEWIAWIYAGTGDTNYNQKFTGRVTMTTDTSTSTAYMELRSLRSDDTAVYYCARHGMTGRGWYFAVWGQGTTVTVSS

SEQ ID NO: 32 - protein, 109 aa, synthetic construct
QAVVTQEPSLTVSPGGTVTLTCRSSTGAVTTSNLANWVQQKPGQAFRGLIGHTNNRAPGVPARFSGSLLGDKAALTLSGAQPEDEAEYYCILWYSNKFVFGGGTKLTVL

SEQ ID NO: 33 - protein, 451 aa, synthetic construct
QVQLVQSGAEVKKPGASVKVSCKASGYTFTSSYISWVRQAPGQGLEWIAWIYAGTGDTNYNQKFTGRVTMTTDTSTSTAYMELRSLRSDDTAVYYCARHGYTGRGWYFAVWGQGTTVTVSSASTKGPSVFPLAPSSKSTSGGTAALGCLVKDYFPEPVTVSWNSGALTSGVHTFPAVLQSSGLYSLSSVVTVPSSSLGTQTYICNVNHKPSNTKVDKKVEPKSCDKTHTCPPCPAPELLGGPSVFLFPPKPKDTLMISRTPEVTCVVVDVSHEDPEVKFNWYVDGVEVHNAKTKPREEQYNSTYRVVSVLTVLHQDWLNGKEYKCKVSNKALPAPIEKTISKAKGQPREPQVYTLPPSREEMTKNQVSLTCLVKGFYPSDIAVEWESNGQPENNYKTTPPVLDSDGSFFLYSKLTVDKSRWQQGNVFSCSVMHEALHNHYTQKSLSLSPGK

SEQ ID NO: 34 - protein, 215 aa, synthetic construct
QAVVTQEPSLTVSPGGTVTLTCRSSTGAVTTSNLANWVQQKPGQAFRGLIGHTNNRAPGVPARFSGSLLGDKAALTLSGAQPEDEAEYYCALWYSNKFVFGGGTKLTVLGQPKAAPSVTLFPPSSEELQANKATLVCLISDFYPGAVTVAWKADSSPVKAGVETTTPSKQSNNKYAASSYLSLTPEQWKSHRSYSCQVTHEGSTVEKTVAPTECS

SEQ ID NO: 35 - protein, 451 aa, synthetic construct; identical to SEQ ID NO: 33

SEQ ID NO: 36 - protein, 215 aa, synthetic construct
QAVVTQEPSLTVSPGGTVTLTCRSSTGAVTTSNYANWVQQKPGQAFRGLIGGTNNRAPGVPARFSGSLLGDKAALTLSGAQPEDEAEYYCILWYSNHFVFGGGTKLTVLGQPKAAPSVTLFPPSSEELQANKATLVCLISDFYPGAVTVAWKADSSPVKAGVETTTPSKQSNNKYAASSYLSLTPEQWKSHRSYSCQVTHEGSTVEKTVAPTECS

SEQ ID NO: 37 - protein, 451 aa, synthetic construct
QVQLVQSGAEVKKPGASVKVSCKASGYTFTSSYISWVRQAPGQGLEWIAWIYAGTGDTNYNQKFTGRVTMTTDTSTSTAYMELRSLRSDDTAVYYCARHGLTGRHWYFAVWGQGTTVTVSSASTKGPSVFPLAPSSKSTSGGTAALGCLVKDYFPEPVTVSWNSGALTSGVHTFPAVLQSSGLYSLSSVVTVPSSSLGTQTYICNVNHKPSNTKVDKKVEPKSCDKTHTCPPCPAPELLGGPSVFLFPPKPKDTLMISRTPEVTCVVVDVSHEDPEVKFNWYVDGVEVHNAKTKPREEQYNSTYRVVSVLTVLHQDWLNGKEYKCKVSNKALPAPIEKTISKAKGQPREPQVYTLPPSREEMTKNQVSLTCLVKGFYPSDIAVEWESNGQPENNYKTTPPVLDSDGSFFLYSKLTVDKSRWQQGNVFSCSVMHEALHNHYTQKSLSLSPGK

SEQ ID NO: 38 - protein, 215 aa, synthetic construct
QAVVTQEPSLTVSPGGTVTLTCRSSTGAVTTSNIANWVQQKPGQAFRGLIGGTNNRGPGVPARFSGSLLGDKAALTLSGAQPEDEAEYYCILWYSNKFVFGGGTKLTVLGQPKAAPSVTLFPPSSEELQANKATLVCLISDFYPGAVTVAWKADSSPVKAGVETTTPSKQSNNKYAASSYLSLTPEQWKSHRSYSCQVTHEGSTVEKTVAPTECS

SEQ ID NO: 39 - protein, 451 aa, synthetic construct
QVQLVQSGAEVKKPGASVKVSCKASGYTFTSSYISWVRQAPGQGLEWIAWIYAGTGDTNYNQKFTGRVTMTTDTSTSTAYMELRSLRSDDTAVYYCARHGMTGRGWYFAVWGQGTTVTVSSASTKGPSVFPLAPSSKSTSGGTAALGCLVKDYFPEPVTVSWNSGALTSGVHTFPAVLQSSGLYSLSSVVTVPSSSLGTQTYICNVNHKPSNTKVDKKVEPKSCDKTHTCPPCPAPELLGGPSVFLFPPKPKDTLMISRTPEVTCVVVDVSHEDPEVKFNWYVDGVEVHNAKTKPREEQYNSTYRVVSVLTVLHQDWLNGKEYKCKVSNKALPAPIEKTISKAKGQPREPQVYTLPPSREEMTKNQVSLTCLVKGFYPSDIAVEWESNGQPENNYKTTPPVLDSDGSFFLYSKLTVDKSRWQQGNVFSCSVMHEALHNHYTQKSLSLSPGK

SEQ ID NO: 40 - protein, 215 aa, synthetic construct
QAVVTQEPSLTVSPGGTVTLTCRSSTGAVTTSNLANWVQQKPGQAFRGLIGHTNNRAPGVPARFSGSLLGDKAALTLSGAQPEDEAEYYCILWYSNKFVFGGGTKLTVLGQPKAAPSVTLFPPSSEELQANKATLVCLISDFYPGAVTVAWKADSSPVKAGVETTTPSKQSNNKYAASSYLSLTPEQWKSHRSYSCQVTHEGSTVEKTVAPTECS

SEQ ID NO: 41 - protein, 330 aa, synthetic construct
ASTKGPSVFPLAPSSKSTSGGTAALGCLVKDYFPEPVTVSWNSGALTSGVHTFPAVLQSSGLYSLSSVVTVPSSSLGTQTYICNVNHKPSNTKVDKKVEPKSCDKTHTCPPCPAPELLGGPSVFLFPPKPKDTLMISRTPEVTCVVVDVSHEDPEVKFNWYVDGVEVHNAKTKPREEQYNSTYRVVSVLTVLHQDWLNGKEYKCKVSNKALPAPIEKTISKAKGQPREPQVYTLPPSREEMTKNQVSLTCLVKGFYPSDIAVEWESNGQPENNYKTTPPVLDSDGSFFLYSKLTVDKSRWQQGNVFSCSVMHEALHNHYTQKSLSLSPGK

SEQ ID NO: 42 - protein, 330 aa, synthetic construct
ASTKGPSVFPLAPSSKSTSGGTAALGCLVKDYFPEPVTVSWNSGALTSGVHTFPAVLQSSGLYSLSSVVTVPSSSLGTQTYICNVNHKPSNTKVDKKVEPKSCDKTHTCPPCPAPEAAGGPSVFLFPPKPKDTLMISRTPEVTCVVVDVSHEDPEVKFNWYVDGVEVHNAKTKPREEQYNSTYRVVSVLTVLHQDWLNGKEYKCKVSNKALPAPIEKTISKAKGQPREPQVYTLPPSREEMTKNQVSLTCLVKGFYPSDIAVEWESNGQPENNYKTTPPVLDSDGSFFLYSKLTVDKSRWQQGNVFSCSVMHEALHNHYTQKSLSLSPGK

SEQ ID NO: 43 - protein, 327 aa, synthetic construct
ASTKGPSVFPLAPCSRSTSESTAALGCLVKDYFPEPVTVSWNSGALTSGVHTFPAVLQSSGLYSLSSVVTVPSSSLGTKTYTCNVDHKPSNTKVDKRVESKYGPPCPPCPAPEFLGGPSVFLFPPKPKDTLMISRTPEVTCVVVDVSQEDPEVQFNWYVDGVEVHNAKTKPREEQFNSTYRVVSVLTVLHQDWLNGKEYKCKVSNKGLPSSIEKTISKAKGQPREPQVYTLPPSQEEMTKNQVSLTCLVKGFYPSDIAVEWESNGQPENNYKTTPPVLDSDGSFFLYSRLTVDKSRWQEGNVFSCSVMHEALHNHYTQKSLSLSLGK

SEQ ID NO: 44 - protein, 106 aa, synthetic construct
GQPKAAPSVTLFPPSSEELQANKATLVCLISDFYPGAVTVAWKADSSPVKAGVETTTPSKQSNNKYAASSYLSLTPEQWKSHRSYSCQVTHEGSTVEKTVAPTECS

SEQ ID NO: 45 - DNA, 1251 bp, synthetic construct
  source 1..1251: mol_type = other DNA
atggctagagctatggcagctgcttggccactgttgttggttgcattgctggtgctctcttggccacctccaggaacaggagatgtggtggtccaggcacctacccaggtccctggtttcctcggggactccgtgaccctcccatgttatctgcaggtgcccaacatggaggtcacacacgtttcacagcttacctgggcccgtcacggggaaagtggctctatggctgtgtttcaccagactcaaggtccttcctatagcgagtcaaagcgactcgagtttgtcgccgccaggctgggagcagaattgaggaacgcttctctgcggatgtttggcctgcgtgtggaagacgagggaaattacacctgcctctttgtcactttccctcagggctcccgttccgtggacatttggctgagggtgctggctaaaccccagaacactgcagaagtgcagaaggtgcagcttaccggcgaacctgtgcccatggctcggtgtgtgtctaccggtggaagaccacctgctcagatcacatggcatagtgacctgggggggatgccaaacacctcacaggtccctggcttcttgtccggtacagtcactgtgacctcactttggatcctggtgccatccagtcaggtggatggcaagaatgtgacatgcaaggtggaacatgagtcatttgagaaaccccaactgctgactgtgaatctgaccgtctactacccacccgaagtgtctatctcaggctacgataataactggtatttgggtcaaaatgaggcaacacttacttgcgatgcccgttccaaccctgaacctaccggatataattggagcaccaccatgggtccactccctccatttgccgtggctcaaggggcccagttgctcattaggcccgtcgataagccaattaacacaacccttatttgcaatgtaactaacgccttgggggccagacaggcagaactgaccgtccaggtgaaggaaggaccaccctcagagcatagcggaatcagcaggaacgcaatcatctttttggtgcttgggattctcgtgtttctgattcttttgggcatcggcatttacttttattggtccaagtgctcccgtgaagtgctgtggcactgccacctgtgcccttcaagtacagagcacgcatctgccagcgctaatgggcacgtgagttattccgctgtatctagagaaaacagttcaagccaggatcctcagaccgagggaacccgc

SEQ ID NO: 46 - DNA, 1251 bp, synthetic construct
  source 1..1251: mol_type = other DNA
atggcaagaacaatggccgctgcctggcctccattgcttttgactctgctcgaattgtcttggccccccccaggaaccggggatatcatcgtccaggcccctacacaagtccctggcttcctgggcgactcagtgaccctgccatgctatcttcaggtccctgggatggaggagacacacgtgagccagcttacatggtcaaggcacggtgaatctggctccatggcagtattccatcagacacagggccccaattactcagaacccaaaaggttggaattcgtcgctgcccgactgggtacagaacttcgtgacgccagtctgagaatgttcggcctgagggtcgaggacgaaggcaactacacttgtctgtttgtgacctttccacagggttctaggtctgtagacatctggttgcgagtcttggcaaagccacagaataccgccgaggtgcagaaggtgcagttgacagggaagccagtccccgtggcacgatgcgtatctactggtgggcggcctcctgcacatatcacatggcactctgatctgggagggatgcctaacacctctcaagcccccggcttcttgagcgggaccgttacagtgacatcactgtggatcttggtgccatcatcccaggttgacggcaagagcgtgacctgcaaagtagagcacgagtcctttgagaagccacagctgctcactgtcaatttgactgtgtattaccctcccgaggtgtccatcagcgggtatgacaacaactggtatctgagccagaatgaagccaccctgacttgcgatgcacgatctaatcccgagccaactggttataactggtctactacaatgggtccattgcccccatttgcagtcgctcagggagcccaactcttgatacggccagtggataaacctatcaatactaccttcatctgtaatgttactaacgctctgggcgctagacaggcagagctcaccgtccaggtgaaggaaggcccacccagtgagccctcaggtatgagctctaacatcattattttcctcatactgggcattgtgatcctcctgactctccttggtatcggcgtgtacttttaccgatctcgctgcagccgggagtttctgtggtgtcaccacttgtcacccagttctgaggagcatgcttctgctagcgccaacggctatatcagttacagcgatgtgagtagggaggcatcaagcagccaggatccacagaccgagggcaccaga

SEQ ID NO: 47 - protein, 8 aa, synthetic construct
GFTFSSSY

SEQ ID NO: 48 - protein, 8 aa, synthetic construct
IYAGTGDT

SEQ ID NO: 49 - protein, 14 aa, synthetic construct
VRHGSTGRGWYFAV

SEQ ID NO: 50 - protein, 8 aa, synthetic construct
TGAVTTSN

SEQ ID NO: 51 - skipped

SEQ ID NO: 52 - protein, 9 aa, synthetic construct
ALWYSNHFV

SEQ ID NO: 53 - protein, 121 aa, synthetic construct
QVQMQQSGAELVKPGASVKLSCKTSGFTFSSSYISWLKQKPGQSLEWIAWIYAGTGDTNYNQKFTGKAQVTVDTSSSTAYMQFSSLTTEDSAIYYCVRHGSTGRGWYFAVWGAGTTVTVSS

SEQ ID NO: 54 - protein, 109 aa, synthetic construct
QAVVTQESALTTSPGETVTLTCRSSTGAVTTSNYANWVQEKPDHLFTGLIGGTNNRAPGVPARFSGSLIGDKAALTITGAQTEDEAIYFCALWYSNHFVFGGGTKLTVL

SEQ ID NO: 55 - protein, 451 aa, synthetic construct
QVQMQQSGAELVKPGASVKLSCKTSGFTFSSSYISWLKQKPGQSLEWIAWIYAGTGDTNYNQKFTGKAQVTVDTSSSTAYMQFSSLTTEDSAIYYCVRHGSTGRGWYFAVWGAGTTVTVSSAKTTAPSVYPLAPVCGDTTGSSVTLGCLVKGYFPEPVTLTWNSGSLSSGVHTFPAVLQSDLYTLSSSVTVTSSTWPSQSITCNVAHPASSTKVDKKIEPRGPTIKPCPPCKCPAPNLLGGPSVFIFPPKIKDVLMISLSPIVTCVVVDVSEDDPDVQISWFVNNVEVHTAQTQTHREDYNSTLRVVSALPIQHQDWMSGKEFKCKVNNKDLPAPIERTISKPKGSVRAPQVYVLPPPEEEMTKKQVTLTCMVTDFMPEDIYVEWTNNGKTELNYKNTEPVLDSDGSYFMYSKLRVEKKNWVERNSYSCSVVHEGLHNHHTTKSFSRTPGK

SEQ ID NO: 56 - protein, 214 aa, synthetic construct
QAVVTQESALTTSPGETVTLTCRSSTGAVTTSNYANWVQEKPDHLFTGLIGGTNNRAPGVPARFSGSLIGDKAALTITGAQTEDEAIYFCALWYSNHFVFGGGTKLTVLQPKSSPSVTLFPPSSEELETNKATLVCTITDFYPGVVTVDWKVDGTPVTQGMETTQPSKQSNNKYMASSYLTLTARAWERHSSYSCQVTHEGHTVEKSLSRADCS

SEQ ID NO: 57 - protein, 8 aa, synthetic construct
GYTFTSSY

SEQ ID NO: 58 - protein, 8 aa, synthetic construct
IYAGTGDT

SEQ ID NO: 59 - protein, 14 aa, synthetic construct
ARHGSTGRGWYFAV

SEQ ID NO: 60 - protein, 8 aa, synthetic construct
TGAVTTSN

SEQ ID NO: 61 - skipped

SEQ ID NO: 62 - protein, 9 aa, synthetic construct
ALWYSNHFV

SEQ ID NO: 63 - protein, 121 aa, synthetic construct
QVQLVQSGAEVKKPGASVKVSCKASGYTFTSSYISWVRQAPGQGLEWIAWIYAGTGDTNYNQKFTGRVTMTTDTSTSTAYMELRSLRSDDTAVYYCARHGSTGRGWYFAVWGQGTTVTVSS

SEQ ID NO: 64 - protein, 109 aa, synthetic construct
QAVVTQEPSLTVSPGGTVTLTCRSSTGAVTTSNYANWVQQKPGQAFRGLIGGTNNRAPGVPARFSGSLLGDKAALTLSGAQPEDEAEYYCALWYSNHFVFGGGTKLTVL

SEQ ID NO: 65 - protein, 451 aa, synthetic construct
QVQLVQSGAEVKKPGASVKVSCKASGYTFTSSYISWVRQAPGQGLEWIAWIYAGTGDTNYNQKFTGRVTMTTDTSTSTAYMELRSLRSDDTAVYYCARHGSTGRGWYFAVWGQGTTVTVSSASTKGPSVFPLAPSSKSTSGGTAALGCLVKDYFPEPVTVSWNSGALTSGVHTFPAVLQSSGLYSLSSVVTVPSSSLGTQTYICNVNHKPSNTKVDKKVEPKSCDKTHTCPPCPAPELLGGPSVFLFPPKPKDTLMISRTPEVTCVVVDVSHEDPEVKFNWYVDGVEVHNAKTKPREEQYNSTYRVVSVLTVLHQDWLNGKEYKCKVSNKALPAPIEKTISKAKGQPREPQVYTLPPSREEMTKNQVSLTCLVKGFYPSDIAVEWESNGQPENNYKTTPPVLDSDGSFFLYSKLTVDKSRWQQGNVFSCSVMHEALHNHYTQKSLSLSPGK

SEQ ID NO: 66 - protein, 215 aa, synthetic construct
QAVVTQEPSLTVSPGGTVTLTCRSSTGAVTTSNYANWVQQKPGQAFRGLIGGTNNRAPGVPARFSGSLLGDKAALTLSGAQPEDEAEYYCALWYSNHFVFGGGTKLTVLGQPKAAPSVTLFPPSSEELQANKATLVCLISDFYPGAVTVAWKADSSPVKAGVETTTPSKQSNNKYAASSYLSLTPEQWKSHRSYSCQVTHEGSTVEKTVAPTECS

SEQ ID NO: 67 - protein, 448 aa, synthetic construct
QVQLVQSGAEVKKPGASVKVSCKASGYTFTSSYISWVRQAPGQGLEWIAWIYAGTGDTNYNQKFTGRVTMTTDTSTSTAYMELRSLRSDDTAVYYCARHGSTGRGWYFAVWGQGTTVTVSSASTKGPSVFPLAPCSRSTSESTAALGCLVKDYFPEPVTVSWNSGALTSGVHTFPAVLQSSGLYSLSSVVTVPSSSLGTKTYTCNVDHKPSNTKVDKRVESKYGPPCPPCPAPEFLGGPSVFLFPPKPKDTLMISRTPEVTCVVVDVSQEDPEVQFNWYVDGVEVHNAKTKPREEQFNSTYRVVSVLTVLHQDWLNGKEYKCKVSNKGLPSSIEKTISKAKGQPREPQVYTLPPSQEEMTKNQVSLTCLVKGFYPSDIAVEWESNGQPENNYKTTPPVLDSDGSFFLYSRLTVDKSRWQEGNVFSCSVMHEALHNHYTQKSLSLSLGK

SEQ ID NO: 68 - protein, 215 aa, synthetic construct; identical to SEQ ID NO: 66

SEQ ID NO: 69 - protein, 451 aa, synthetic construct
QVQMQQSGAELVKPGASVKLSCKTSGFTFSSSYISWLKQKPGQSLEWIAWIYAGTGDTNYNQKFTGKAQVTVDTSSSTAYMQFSSLTTEDSAIYYCVRHGSTGRGWYFAVWGAGTTVTVSSASTKGPSVFPLAPSSKSTSGGTAALGCLVKDYFPEPVTVSWNSGALTSGVHTFPAVLQSSGLYSLSSVVTVPSSSLGTQTYICNVNHKPSNTKVDKKVEPKSCDKTHTCPPCPAPELLGGPSVFLFPPKPKDTLMISRTPEVTCVVVDVSHEDPEVKFNWYVDGVEVHNAKTKPREEQYNSTYRVVSVLTVLHQDWLNGKEYKCKVSNKALPAPIEKTISKAKGQPREPQVYTLPPSREEMTKNQVSLTCLVKGFYPSDIAVEWESNGQPENNYKTTPPVLDSDGSFFLYSKLTVDKSRWQQGNVFSCSVMHEALHNHYTQKSLSLSPGK

SEQ ID NO: 70 - protein, 215 aa, synthetic construct
QAVVTQESALTTSPGETVTLTCRSSTGAVTTSNYANWVQEKPDHLFTGLIGGTNNRAPGVPARFSGSLIGDKAALTITGAQTEDEAIYFCALWYSNHFVFGGGTKLTVLGQPKAAPSVTLFPPSSEELQANKATLVCLISDFYPGAVTVAWKADSSPVKAGVETTTPSKQSNNKYAASSYLSLTPEQWKSHRSYSCQVTHEGSTVEKTVAPTECS

SEQ ID NO: 71 - protein, 448 aa, synthetic construct
QVQMQQSGAELVKPGASVKLSCKTSGFTFSSSYISWLKQKPGQSLEWIAWIYAGTGDTNYNQKFTGKAQVTVDTSSSTAYMQFSSLTTEDSAIYYCVRHGSTGRGWYFAVWGAGTTVTVSSASTKGPSVFPLAPCSRSTSESTAALGCLVKDYFPEPVTVSWNSGALTSGVHTFPAVLQSSGLYSLSSVVTVPSSSLGTKTYTCNVDHKPSNTKVDKRVESKYGPPCPPCPAPEFLGGPSVFLFPPKPKDTLMISRTPEVTCVVVDVSQEDPEVQFNWYVDGVEVHNAKTKPREEQFNSTYRVVSVLTVLHQDWLNGKEYKCKVSNKGLPSSIEKTISKAKGQPREPQVYTLPPSQEEMTKNQVSLTCLVKGFYPSDIAVEWESNGQPENNYKTTPPVLDSDGSFFLYSRLTVDKSRWQEGNVFSCSVMHEALHNHYTQKSLSLSLGK

SEQ ID NO: 72 - protein, 215 aa, synthetic construct; identical to SEQ ID NO: 70

SEQ ID NO: 73 - protein, 417 aa, Homo sapiens
MARAMAAAWPLLLVALLVLSWPPPGTGDVVVQAPTQVPGFLGDSVTLPCYLQVPNMEVTHVSQLTWARHGESGSMAVFHQTQGPSYSESKRLEFVAARLGAELRNASLRMFGLRVEDEGNYTCLFVTFPQGSRSVDIWLRVLAKPQNTAEVQKVQLTGEPVPMARCVSTGGRPPAQITWHSDLGGMPNTSQVPGFLSGTVTVTSLWILVPSSQVDGKNVTCKVEHESFEKPQLLTVNLTVYYPPEVSISGYDNNWYLGQNEATLTCDARSNPEPTGYNWSTTMGPLPPFAVAQGAQLLIRPVDKPINTTLICNVTNALGARQAELTVQVKEGPPSEHSGISRNAIIFLVLGILVFLILLGIGIYFYWSKCSREVLWHCHLCPSSTEHASASANGHVSYSAVSRENSSSQDPQTEGTR

SEQ ID NO: 74 - protein, 417 aa, synthetic construct
MARTMAAAWPPLLLTLLELSWPPPGTGDIIVQAPTQVPGFLGDSVTLPCYLQVPGMEETHVSQLTWSRHGESGSMAVFHQTQGPNYSEPKRLEFVAARLGTELRDASLRMFGLRVEDEGNYTCLFVTFPQGSRSVDIWLRVLAKPQNTAEVQKVQLTGKPVPVARCVSTGGRPPAHITWHSDLGGMPNTSQAPGFLSGTVTVTSLWILVPSSQVDGKSVTCKVEHESFEKPQLLTVNLTVYYPPEVSISGYDNNWYLSQNEATLTCDARSNPEPTGYNWSTTMGPLPPFAVAQGAQLLIRPVDKPINTTFICNVTNALGARQAELTVQVKEGPPSEPSGMSSNIIIFLILGIVILLTLLGIGVYFYRSRCSREFLWCHHLSPSSEEHASASANGYISYSDVSREASSSQDPQTEGTR

SEQ ID NO: 75 - protein, 570 aa, synthetic construct
MARAMAAAWPLLLVALLVLSWPPPGTGDVVVQAPTQVPGFLGDSVTLPCYLQVPNMEVTHVSQLTWARHGESGSMAVFHQTQGPSYSESKRLEFVAARLGAELRNASLRMFGLRVEDEGNYTCLFVTFPQGSRSVDIWLRVLAKPQNTAEVQKVQLTGEPVPMARCVSTGGRPPAQITWHSDLGGMPNTSQVPGFLSGTVTVTSLWILVPSSQVDGKNVTCKVEHESFEKPQLLTVNLTVYYPPEVSISGYDNNWYLGQNEATLTCDARSNPEPTGYNWSTTMGPLPPFAVAQGAQLLIRPVDKPINTTLICNVTNALGARQAELTVQVKEGPPSEHSGPKSCDKTHTCPPCPAPELLGGPSVFLFPPKPKDTLMISRTPEVTCVVVDVSHEDPEVKFNWYVDGVEVHNAKTKPREEQYNSTYRVVSVLTVLHQDWLNGKEYKCKVSNKALPAPIEKTISKAKGQPREPQVYTLPPSREEMTKNQVSLTCLVKGFYPSDIAVEWESNGQPENNYKTTPPVLDSDGSFFLYSKLTVDKSRWQQGNVFSCSVMHEALHNHYTQKSLSLSPGK

SEQ ID NO: 76 - protein, 362 aa, synthetic construct
METDTLLLWVLLLWVPGSTGEFMMTGTIETTGNISAEKGGSIILQCHLSSTTAQVTQVNWEQQDQLLAICNADLGWHISPSFKDRVAPGPGLGLTLQSLTVNDTGEYFCIYHTYPDGTYTGRIFLEVLELEPKSCDKTHTCPPCPAPELLGGPSVFLFPPKPKDTLMISRTPEVTCVVVDVSHEDPEVKFNWYVDGVEVHNAKTKPREEQYNSTYRVVSVLTVLHQDWLNGKEYKCKVSNKALPAPIEKTISKAKGQPREPQVYTLPPSRDELTKNQVSLTCLVKGFYPSDIAVEWESNGQPENNYKTTPPVLDSDGSFFLYSKLTVDKSRWQQGNVFSCSVMHEALHNHYTQKSLSLSPGK

SEQ ID NO: 77 - protein, 492 aa, synthetic construct
MEKKWKYCAVYYIIQIHFVKGVWEKTVNTEENVYATLGSDVNLTCQTQTVGFFVQMQWSKVTNKIDLIAVYHPQYGFYCAYGRPCESLVTFTETPENGSKWTLHLRNMSCSVSGRYECMLVLYPEGIQTKIYNLLIQTHVTADEWNSNHTIEIEINQTLEIPCFQNSSSKISSEFTYAWSVENSSTDSWVLLSKGIKEDNGTQETLISQNHLISNSTLLKDRVKLGTDYRLHLSPVQIFDDGRKFSCHIRVGPNKILRSSTPKSCDKTHTCPPCPAPELLGGPSVFLFPPKPKDTLMISRTPEVTCVVVDVSHEDPEVKFNWYVDGVEVHNAKTKPREEQYNSTYRVVSVLTVLHQDWLNGKEYKCKVSNKALPAPIEKTISKAKGQPREPQVYTLPPSREEMTKNQVSLTCLVKGFYPSDIAVEWESNGQPENNYKTTPPVLDSDGSFFLYSKLTVDKSRWQQGNVFSCSVMHEALHNHYTQKSLSLSPGK

SEQ ID NO: 78 - protein, 486 aa, synthetic construct
MGWSCIILFLVATATGVHSEEVLWHTSVPFAENMSLECVYPSMGILTQVEWFKIGTQQDSIAIFSPTHGMVIRKPYAERVYFLNSTMASNNMTLFFRNASEDDVGYYSCSLYTYPQGTWQKVIQVVQSDSFEAAVPSNSHIVSEPGKNVTLTCQPQMTWPVQAVRWEKIQPRQIDLLTYCNLVHGRNFTSKFPRQIVSNCSHGRWSVIVIPDVTVSDSGLYRCYLQASAGENETFVMRLTVAEGKTDNQYTLFVAPKSCDKTHTCPPCPAPELLGGPSVFLFPPKPKDTLMISRTPEVTCVVVDVSHEDPEVKFNWYVDGVEVHNAKTKPREEQYNSTYRVVSVLTVLHQDWLNGKEYKCKVSNKALPAPIEKTISKAKGQPREPQVYTLPPSRDELTKNQVSLTCLVKGFYPSDIAVEWESNGQPENNYKTTPPVLDSDGSFFLYSKLTVDKSRWQQGNVFSCSVMHEALHNHYTQKSLSLSPGK

SEQ ID NO: 79 - protein, 449 aa, synthetic construct
QVQLVQSGAEVKKPGASVKVSCKATGYTFSNYWIEWVRQAPGQGLEWIGEIFPGSGRINFNEKFKGRVTFTADTSISTTYMELSRLRSDDTAVYYCARTKIYGNSFDYWGQGTLVTVSSASTKGPSVFPLAPSSKSTSGGTAALGCLVKDYFPEPVTVSWNSGALTSGVHTFPAVLQSSGLYSLSSVVTVPSSSLGTQTYICNVNHKPSNTKVDKKVEPKSCDKTHTCPPCPAPELLGGPSVFLFPPKPKDTLMISRTPEVTCVVVDVSHEDPEVKFNWYVDGVEVHNAKTKPREEQYNSTYRVVSVLTVLHQDWLNGKEYKCKVSNKALPAPIEKTISKAKGQPREPQVYTLPPSREEMTKNQVSLTCLVKGFYPSDIAVEWESNGQPENNYKTTPPVLDSDGSFFLYSKLTVDKSRWQQGNVFSCSVMHEALHNHYTQKSLSLSPGK

SEQ ID NO: 80 - protein, 446 aa, synthetic construct
QVQLVQSGAEVKKPGASVKVSCKATGYTFSNYWIEWVRQAPGQGLEWIGEIFPGSGRINFNEKFKGRVTFTADTSISTTYMELSRLRSDDTAVYYCARTKIYGNSFDYWGQGTLVTVSSASTKGPSVFPLAPCSRSTSESTAALGCLVKDYFPEPVTVSWNSGALTSGVHTFPAVLQSSGLYSLSSVVTVPSSSLGTKTYTCNVDHKPSNTKVDKRVESKYGPPCPPCPAPEFLGGPSVFLFPPKPKDTLMISRTPEVTCVVVDVSQEDPEVQFNWYVDGVEVHNAKTKPREEQFNSTYRVVSVLTVLHQDWLNGKEYKCKVSNKGLPSSIEKTISKAKGQPREPQVYTLPPSQEEMTKNQVSLTCLVKGFYPSDIAVEWESNGQPENNYKTTPPVLDSDGSFFLYSRLTVDKSRWQEGNVFSCSVMHEALHNHYTQKSLSLSLGK

SEQ ID NO: 81 - protein, 214 aa, synthetic construct
DIQMTQSPSSLSASVGDRVTITCKASQDVGTAVVWYQQKPGKAPKLLIYWASSRHEGVPDRFSGSGSGTDFTLTISSLQPEDFADYFCQQYSRYPLTFGQGTKLEIKRTVAAPSVFIFPPSDEQLKSGTASVVCLLNNFYPREAKVQWKVDNALQSGNSQESVTEQDSKDSTYSLSSTLTLSKADYEKHKVYACEVTHQGLSSPVTKSFNRGEC